European Patent Application EP 4 130 732 A1, published February 8, 2023. Title: METHOD FOR ANALYZING IMPURITY MOLECULES IN COMPOSITIONS CONTAINING MULTISPECIFIC ANTIGEN BINDING MOLECULES. Applicant: CHUGAI SEIYAKU KABUSHIKI KAISHA. The sequence listing filed with the application follows.

SEQUENCE LISTING (21 sequences)

SEQ ID NO: 1 - protein, 122 aa, Artificial Sequence
  VH region
QVQLVESGGGLVQPGGSLRLSCAASGFTFSYYDIQWVRQAPGKGLEWVSSISPSGQSTYYRREVKGRFTISRDNSKNTLYLQMNSLRAEDTAVYYCARRTGREEGGWIFDYWGQGTLVTVSS

SEQ ID NO: 2 - protein, 107 aa, Artificial Sequence
  VL region
EIVLTQSPATLSVSPGERATLSCRASRSVRRELAWYQQKPGQAPELLIYGASTRETGIPARFSGSGSGTDFTLTINSLEAEDAATYYCQQYRDPPGTFGGGTKVEIK

SEQ ID NO: 3 - protein, 325 aa, Artificial Sequence
  CH region
ASTKGPSVFPLAPCSRSTSESTAALGCLVKDYFPEPVTVSWNSGALTSGVHTFPAVLKSSGLYSLSSVVTVPSSSLGTQTYTCNVDHKPSNTKVDKRVESKYGPPCPPCPAPEFLGGPSVFLFPPKPKDTLMISRTPEVTCVVVDVSQEDPEVQFNWYVDGVEVHNAKTKPREEQYNSTYRVVSVLTVLHQDWLNGKEYKCKVSNKGLPSSIEKTISKAKGQPREPQVYTLPPSQKEMTKNQVSLTCLVKGFYPSDIAVEWESNGQPENNYKTTPPVLDSDGSFFLYSKLTVDKSRWQEGNVFSCSVLHEALHAHYTRKELSLSP

SEQ ID NO: 4 - protein, 107 aa, Artificial Sequence
  CL region
RTVAAPSVFIFPPSDEQLKSGTAEVVCLLNNFYPREAKVQWKVDNALQSGNSQESVTEQDSKDSTYSLSSTLELSKADYEKHKVYACEVTHQGLSSPVTKSFNRGEC

SEQ ID NO: 5 - protein, 119 aa, Artificial Sequence
  VH region
QVQLVQSGSELKKPGASVKVSCKASGYTFTQNNMDWVRQAPGQGLEWMGDINTRSGGVIYNEEFQDRLIMTVDKSTDTAYMELSSLRSEDTATYHCARRKSYGYYLDVWGEGTLVTVSS

SEQ ID NO: 6 - protein, 107 aa, Artificial Sequence
  VL region
SYVLTQPVSVSVALGQTATITCEGEQIGSKEVHWYHQRPGQAPILVMFRDARRPSGIPERLSGSNSGNTASLTISGAEAGDEGDYYCQVWDSSSYTVFGGGTKVTVV

SEQ ID NO: 7 - protein, 325 aa, Artificial Sequence
  CH region
ASTKGPSVFPLAPCSRSTSESTAALGCLVEDYFPEPVTVSWNSGALTSGVHTFPAVLESSGLYSLSSVVTVPSSSLGTQTYTCNVDHKPSNTKVDKRVESKYGPPCPPCPAPEFLGGPSVFLFPPKPKDTLMISRTPEVTCVVVDVSQEDPEVQFNWYVDGVEVHNAKTKPREEQYNSTYRVVSVLTVLHQDWLNGKEYKCKVSNKGLPSSIEKTISKAKGQPREPQVYTLPPSQEEMTKNQVSLTCLVKGFYPSDIAVEWESNGQPENNYKTTPPVLDSDGSFFLYSKLTVDKSRWQEGNVFSCSVLHEALHAHYTREELSLSP

SEQ ID NO: 8 - protein, 106 aa, Artificial Sequence
  CL region
GQPKAAPSVTLFPPSSEELQANKAKLVCLISDFYPGAVTVAWKADSSPVKAGVETTTPSKQSNNKYAASSYLKLTPEQWKSHRSYSCQVTHEGSTVEKTVAPTECS

SEQ ID NO: 9 - protein, 116 aa, Artificial Sequence
  VH region
QDQLVQSGAEVKKPGASVKVSCKASGFNIKDTYIQWVRQAPGQGLEWMGRIDPLRKQTKYREKFEGRVTITADTSTNTAYMELSSLRSEDTAVYYCVRSGREFDYWGQGTLVTVSS

SEQ ID NO: 10 - protein, 106 aa, Artificial Sequence
  VL region
DIQMTQSPSSLSASVGDRVTITCRASQDIHKYIAWYQQKPGQAPRLLIQYTSTLQPGVPSRFSGSGSGTDYTFTISSLQPEDIATYYCLQYEQLRTFGGGTKVEIK

SEQ ID NO: 11 - protein, 328 aa, Artificial Sequence
  CH region
ASTKGPSVFPLAPSSKSTSGGTAALGCLVKDYFPEPVTVSWNSGALTSGVHTFPAVLQSSGLYSLSSVVTVPSSSLGTQTYICNVNHKPSNTKVDKKVEPKSCDKTHTCPPCPAPELRGGPKVFLFPPKPKDTLMISRTPEVTCVVVDVSHEDPEVKFNWYVDGVEVHNAKTKPREEQYASTYRVVSVLTVLHQDWLNGKEYKCKVSNKALPAPIEKTISKAKGQPREPQVYTLPPSRKEMTKNQVSLTCLVKGFYPSDIAVEWESNGQPENNYKTTPPYLDSDGSFFLYSKLTVDKSRWQQGNVFSCSVMHEALHNHYTQKSLSLSP

SEQ ID NO: 12 - protein, 107 aa, Artificial Sequence [sequence omitted]

SEQ ID NO: 13 - protein, 115 aa, Artificial Sequence
  VH region
QVQLVQSGAEVKKPGASVTVSCKASGYTFTDYEMHWIRQPPGEGLEWIGAIDGPTPDTAYSEKFKGRVTLTADKSTSTAYMELSSLTSEDTAVYYCTRFYSYTYWGQGTLVTVSS

SEQ ID NO: 14 - protein, 112 aa, Artificial Sequence
  VL region
DIVMTQSPLSLPVTPGEPASISCRSSQPLVHSNRNTYLHWYQQKPGQAPRLLIYKVSNRFSGVPDRFSGSGSGTDFTLKISRVEAEDVGVYYCGQGTQVPYTFGQGTKLEIK

SEQ ID NO: 15 - protein, 328 aa, Artificial Sequence
  CH region
ASTKGPSVFPLAPSSKSTSGGTAALGCLVKDYFPEPVTVSWNSGALTSGVHTFPAVLQSSGLYSLSSVVTVPSSSLGTQTYICNVNHKPSNTKVDKKVEPKSCDKTHTCPPCPAPELRGGPKVFLFPPKPKDTLMISRTPEVTCVVVDVSHEDPEVKFNWYVDGVEVHNAKTKPREEQYASTYRVVSVLTVLHQDWLNGKEYKCKVSNKALPAPIEKTISKAKGQPREPQVYTLPPSREEMTKNQVSLTCLVKGFYPSDIAVEWESNGQPENNYKTTPPYLDSDGSFFLYSKLTVDKSRWQQGNVFSCSVMHEALHNHYTQESLSLSP

SEQ ID NO: 16 - protein, 107 aa, Artificial Sequence [sequence omitted]

SEQ ID NO: 17 - protein, 119 aa, Artificial Sequence [sequence omitted]

SEQ ID NO: 18 - protein, 107 aa, Artificial Sequence [sequence omitted]

SEQ ID NO: 19 - protein, 107 aa, Artificial Sequence [sequence omitted]

SEQ ID NO: 20 - protein, 116 aa, Artificial Sequence
  VH region
QVQLQQSGPQLVRPGASVKISCKASGYSFTSYWMHWVNQRPGQGLEWIGMIDPSYSETRLNQKFKDKATLTVDKSSSTAYMQLSSPTSEDSAVYYCALYGNYFDYWGQGTTLTVSS

SEQ ID NO: 21 - protein, 107 aa, Artificial Sequence
  VL region
DIQMTQSSSSFSVSLGDRVTITCKASEDIYNRLAWYQQKPGNAPRLLISGATSLETGVPSRFSGSGSGKDYTLSITSLQTEDVATYYCQQYWSTPYTFGGGTKLEVK